European Patent Application EP 4 483 954 A1, published January 1, 2025. Title: Substituted thieno [3,2-b]pyridines as inhibitors of protein kinases. Applicant: Masarykova univerzita. Application EP. The sequence listing filed with the application follows.

SEQUENCE LISTING (4 sequences)

SEQ ID NO: 1 - protein, 15 aa, synthetic construct
RRRFRPASPLRGPPK

SEQ ID NO: 2 - protein, 26 aa, synthetic construct
YRRAAVPPSPSLSRHSSPHQSEDEEE

SEQ ID NO: 3 - protein, 11 aa, synthetic construct
RARTLSFAEPG

SEQ ID NO: 4 - protein, 9 aa, synthetic construct
KKRNRTLTV